European Patent Application EP 4 778 591 A2, published July 22, 2026. Title: ANTI-COMPLEMENT FACTOR C1Q FAB FRAGMENTS AND USES THEREOF. Applicant: ANNEXON, INC. Application EP. The sequence listing filed with the application follows.

SEQUENCE LISTING (12 sequences)

SEQ ID NO: 1 - protein, 229 aa, synthetic construct
QVQLVQSGAELKKPGASVKVSCKSSGYHFTSYWMHWVKQAPGQGLEWIGVIHPNSGSINYNEKFESRVTITVDKSTSTAYMELSSLRSEDTAVYYCAGERDSTEVLPMDYWGQGTTVTVSSASTKGPSVFPLAPSSKSTSGGTAALGCLVKDYFPEPVTVSWNSGALTSGVHTFPAVLQSSGLYSLSSVVTVPSSSLGTQTYICNVNHKPSNTKVDKKVEPKSCDKTHT

SEQ ID NO: 2 - protein, 214 aa, synthetic construct
DVQITQSPSSLSASLGERATINCRASKSINKYLAWYQQKPGKAPKLLIYSGSTLQSGIPARFSGSGSGTDFTLTISSLEPEDFAMYYCQQHNEYPLTFGQGTKLEIKRTVAAPSVFIFPPSDEQLKSGTASVVCLLNNFYPREAKVQWKVDNALQSGNSQESVTEQDSKDSTYSLSSTLTLSKADYEKHKVYACEVTHQGLSSPVTKSFNRGEC

SEQ ID NO: 3 - DNA, 687 bp, synthetic construct
  source 1..687: mol_type = other DNA
caggtgcagctggtgcagtcaggggctgagctgaagaagcctggggcttcagtgaaggtttcctgcaagtcttctggctaccatttcaccagctactggatgcactgggtgaagcaggcccctggacaaggccttgagtggattggagtgattcatcctaatagtggtagtattaactacaatgagaagttcgagagcagagtcacaattactgtagacaaatccaccagcacagcctacatggagctcagcagcctgagatctgaggacacggcggtctattattgtgcaggagagagagattctacggaggttctccctatggactactggggtcaaggaaccacggtcaccgtctcctcagcgtccaccaaaggcccgtccgtgtttccgctggcgccgtcctccaaatccacctccggcggcaccgcggcgctgggctgcctggtgaaagattattttccggaaccggtgaccgtgtcctggaattccggcgcgctgacctccggcgtgcatacctttccggcggtgctgcagtcctccggcctgtattccctgtcctccgtggtgaccgtgccgtcctcctccctgggcacccagacctatatttgcaatgtgaatcataaaccgtccaataccaaagtggataaaaaagtggaaccgaaatcctgcgataaaacccatacc

SEQ ID NO: 4 - DNA, 645 bp, synthetic construct
  source 1..645: mol_type = other DNA
gatgtccagatcacacagtctccatcttccctttctgcatctctcggagaaagagctactattaattgcagggcaagtaagagcattaacaaatacttagcctggtatcaacagaaacctgggaaagctcctaagctccttatctactctggctccactttgcaatctggaattccagcaaggttcagtggcagtggatctggtacagatttcactctcaccatcagtagcctggagcctgaagattttgcaatgtattactgtcaacaacataatgaatacccgctcacgttcggtcaggggaccaagctggagatcaaacgaactgtggctgcaccatctgtcttcatcttcccgccatctgatgagcagttgaaatctggaactgcctctgttgtgtgcctgctgaataacttctatcccagagaggccaaagtacagtggaaggtggataacgccctccaatcgggtaactcccaggagagtgtcacagagcaggacagcaaggacagcacctacagcctcagcagcaccctgacgctgagcaaagcagactacgagaaacacaaagtctacgcctgcgaagtcacccatcagggcctgagctcgcccgtcacaaagagcttcaacaggggagagtgttag

SEQ ID NO: 5 - protein, 121 aa, synthetic construct [sequence omitted]

SEQ ID NO: 6 - protein, 121 aa, synthetic construct [sequence omitted]

SEQ ID NO: 7 - protein, 121 aa, synthetic construct
QVQLVQSGAELKKPGASVKVSCKSSGYHFTSYWMHWVKQAPGQGLEWIGVIHPNSGSINYNEKFESRVTITVDKSTSTAYMELSSLRSEDTAVYYCAGERDSTEVLPMDYWGQGTTVTVSS

SEQ ID NO: 8 - protein, 121 aa, synthetic construct [sequence omitted]

SEQ ID NO: 9 - protein, 107 aa, synthetic construct [sequence omitted]

SEQ ID NO: 10 - protein, 107 aa, synthetic construct [sequence omitted]

SEQ ID NO: 11 - protein, 107 aa, synthetic construct
DVQITQSPSSLSASLGERATINCRASKSINKYLAWYQQKPGKAPKLLIYSGSTLQSGIPARFSGSGSGTDFTLTISSLEPEDFAMYYCQQHNEYPLTFGQGTKLEIK

SEQ ID NO: 12 - protein, 107 aa, synthetic construct [sequence omitted]